European Patent Application EP 4 166 649 A1, published April 19, 2023. Title: ORAL RECOMBINANT YEAST FOR EXPRESSING S PROTEIN OF NOVEL CORONAVIRUS, PREPARATION THEREFOR, AND APPLICATION THEREOF. Applicant: TIANJIN UNIVERSITY. The sequence listing filed with the application follows.

SEQUENCE LISTING (7 sequences)

SEQ ID NO: 1 - protein, 702 aa, Artificial Synthesis
MKCTLKSFTVEKGIYQTSNFRVQPTESIVRFPNITNLCPFGEVFNATRFASVYAWNRKRISNCVADYSVLYNSASFSTFKCYGVSPTKLNDLCFTNVYADSFVIRGDEVRQIAPGQTGKIADYNYKLPDDFTGCVIAWNSNNLDSKVGGNYNYLYRLFRKSNLKPFERDISTEIYQAGSTPCNGVEGFNCYFPLQSYGFQPTNGVGYQPYRVVVLSFELLHAPATVCGPKKSTNLVKNKCVNFNFNGLTGTGVLTESNKKFLPFQQFGRDIADTTDAVRDPQTLEILDITPCSFGGVSVITPGTNTSNQVAVLYQDVNCTEVPVAIHADQLTPTWRVYSTGSNVFQTRAGCLIGAEHVNNSYECDIPIGAGICASYQTQTNSPRRARSVASQSIIAYTMSLGAENSVAYSNNSIAIPTNFTISVTTEILPVSMTKTSVDCTMYICGDSTECSNLLLQYGSFCTQLNRALTGIAVEQDKNTQEVFAQVKQIYKTPPIKDFGGFNFSQILPDPSKPSKRSFIEDLLFNKVTLADAGFIKQYGDCLGDIAARDLICAQKFNGLTVLPPLLTDEMIAQYTSALLAGTITSGWTFGAGAALQIPFAMQMAYRFNGIGVTQNVLYENQKLIANQFNSAIGKIQDSLSSTASALGKLQDVVNQNAQALNTLVKQLSSNFGAISSVLNDILSRLDKVEAEVQIDRLITGR

SEQ ID NO: 2 - DNA, 2106 bp, Artificial Synthesis
atgaagtgtacgttgaaatccttcactgtagaaaaaggaatctatcaaacttctaactttagagtccaaccaacagaatctattgttagatttcctaatattacaaacttgtgcccttttggtgaagtttttaacgccaccagatttgcatctgtttatgcttggaacaggaagagaatcagcaactgtgttgctgattattctgtcctatataattccgcatcattttccacttttaagtgttatggagtgtctcctactaaattaaatgatctctgctttactaatgtctatgcagattcatttgtaattagaggtgatgaagtcagacaaatcgctccagggcaaactggaaagattgctgattataattataaattaccagatgattttacaggctgcgttatagcttggaattctaacaatcttgattctaaggttggtggtaattataattacctgtatagattgtttaggaagtctaatctcaaaccttttgagagagatatttcaactgaaatctatcaggccggtagcacaccttgtaatggtgttgaaggttttaattgttactttcctttacaatcatatggtttccaacccactaatggtgttggttaccaaccatacagagtagtagtactttcttttgaacttctacatgcaccagcaactgtttgtggacctaaaaagtctactaatttggttaaaaacaaatgtgtcaatttcaacttcaatggtttaacaggcacaggtgttcttactgagtctaacaaaaagtttctgcctttccaacaatttggcagagacattgctgacactactgatgctgtccgtgatccacagacacttgagattcttgacattacaccatgttcttttggtggtgtcagtgttataacaccaggaacaaatacttctaaccaggttgctgttctttatcaggatgttaactgcacagaagtccctgttgctattcatgcagatcaacttactcctacttggcgtgtttattctacaggttctaatgtttttcaaacacgtgcaggctgtttaataggggctgaacatgtcaacaactcatatgagtgtgacatacccattggtgcaggtatatgcgctagttatcagactcagactaattctcctcggcgggcacgtagtgtagctagtcaatccatcattgcctacactatgtcacttggtgcagaaaattcagttgcttactctaataactctattgccatacccacaaattttactattagtgttaccacagaaattctaccagtgtctatgaccaagacatcagtagattgtacaatgtacatttgtggtgattcaactgaatgcagcaatcttttgttgcaatatggcagtttttgtacacaattaaaccgtgctttaactggaatagctgttgaacaagacaaaaacacccaagaagtttttgcacaagtcaaacaaatttacaaaacaccaccaattaaagattttggtggttttaatttttcacaaatattaccagatccatcaaaaccaagcaagaggtcatttattgaagatctacttttcaayaaagtgacacttgcagatgctggcttcatcaaacaatatggtgattgccttggtgatattgctgctagagacctcatttgtgcacaaaagtttaacggccttactgttttgccacctttgctcacagatgaaatgattgctcaatacacttctgcactgttagcgggtacaatcacttctggttggacctttggtgcaggtgctgcattacaaataccatttgctatgcaaatggcttataggtttaatggtattggagttacacagaatgttctctatgagaaccaaaaattgattgccaaccaatttaatagtgctattggcaaaattcaagactcactttcttccacagcaagtgcacttggaaaacttcaagatgtggtcaaccaaaatgcacaagctttaaacacgcttgttaaacaacttagctccaattttggtgcaatttcaagtgttttaaatgatatcctttcacgtcttgacaaagttgaggctgaagtgcaaattgataggttgatcacaggcaga

SEQ ID NO: 3 - DNA, 8449 bp, Artificial Synthesis
agggcctcgtgatacgcctatttttataggttaatgtcatgataataatggtttcttaggacggatcgcttgcctgtaacttacacgcgcctcgtatcttttaatgatggaataatttgggaatttactctgtgtttatttatttttatgttttgtatttggattttagaaagtaaataaagaaggtagaagagttacggaatgaagaaaaaaaaataaacaaaggtttaaaaaatttcaacaaaaagcgtactttacatatatatttattagacaagaaaagcagattaaatagatatacattcgattaacgataagtaaaatgtaaaatcacaggattttcgtgtgtggtcttctacacagacaagatgaaacaattcggcattaatacctgagagcaggaagagcaagataaaaggtagtatttgttggcgatccccctagagtcttttacatcttcggaaaacaaaaactattttttctttaatttctttttttactttctatttttaatttatatatttatattaaaaaatttaaattataattatttttatagcacgtgatgaaaaggacccaggtggcacttttcggggaaatgtgcgcggaacccctatttgtttatttttctaaatacattcaaatatgtatccgctcatgagacaataaccctgataaatgcttcaataatattgaaaaaggaagagtatgagtattcaacatttccgtgtcgcccttattcccttttttgcggcattttgccttcctgtttttgctcacccagaaacgctggtgaaagtaaaagatgctgaagatcagttgggtgcacgagtgggttacatcgaactggatctcaacagcggtaagatccttgagagttttcgccccgaagaacgttttccaatgatgagcacttttaaagttctgctatgtggcgcggtattatcccgtattgacgccgggcaagagcaactcggtcgccgcatacactattctcagaatgacttggttgagtactcaccagtcacagaaaagcatcttacggatggcatgacagtaagagaattatgcagtgctgccataaccatgagtgataacactgcggccaacttacttctgacaacgatcggaggaccgaaggagctaaccgcttttttgcacaacatgggggatcatgtaactcgccttgatcgttgggaaccggagctgaatgaagccataccaaacgacgagcgtgacaccacgatgcctgtagcaatggcaacaacgttgcgcaaactattaactggcgaactacttactctagcttcccggcaacaattaatagactggatggaggcggataaagttgcaggaccacttctgcgctcggcccttccggctggctggtttattgctgataaatctggagccggtgagcgtggtagtcgcggtatcattgcagcactggggccagatggtaagccctcccgtatcgtagttatctacacgacggggagtcaggcaactatggatgaacgaaatagacagatcgctgagataggtgcctcactgattaagcattggtaactgtcagaccaagtttactcatatatactttagattgatttaaaacttcatttttaatttaaaaggatctaggtgaagatcctttttgataatctcatgaccaaaatcccttaacgtgagttttcgttccactgagcgtcagaccccgtagaaaagatcaaaggatcttcttgagatcctttttttctgcgcgtaatctgctgcttgcaaacaaaaaaaccaccgctaccagcggtggtttgtttgccggatcaagagctaccaactctttttccgaaggtaactggcttcagcagagcgcagataccaaatactgtccttctagtgtagccgtagttaggccaccacttcaagaactctgtagcaccgcctacatacctcgctctgctaatcctgttaccagtggctgctgccagtggcgataagtcgtgtcttaccgggttggactcaagacgatagttaccggataaggcgcagcggtcgggctgaacggggggttcgtgcacacagcccagcttggagcgaacgacctacaccgaactgagatacctacagcgtgagctatgagaaagcgccacgcttcccgaagggagaaaggcggacaggtatccggtaagcggcagggtcggaacaggagagcgcacgagggagcttccagggggaaacgcctggtatctttatagtcctgtcgggtttcgccacctctgacttgagcgtcgatttttgtgatgctcgtcaggggggcggagcctatggaaaaacgccagcaacgcggcctttttacggttcctggccttttgctggccttttgctcacatgttctttcctgcgttatcccctgattctgtggataaccgtattaccgcctttgagtgagctgataccgctcgccgcagccgaacgaccgagcgcagcgagtcagtgagcgaggaagcggaagagcgcccaatacgcaaaccgcctctccccgcgcgttggccgattcattaatgcagctggcacgacaggtttcccgactggaaagcgggcagtgagcgcaacgcaattaatgtgagttacctcactcattaggcaccccaggctttacactttatgcttccggctcctatgttgtgtggaattgtgagcggataacaatttcacacaggaaacagctatgaccatgattacgccaagcgcgcaattaaccctcactaaagggaacaaaagctggagctccaccgcggtggcggccgcgaataccccgggtcgagaggtctcggttggcagtgactcggtctctacctggcttcattatcaatactgccatttcaaagaatacgtaaataattaatagtagtgattttcctaactttatttagtcaaaaaattagccttttaattctgctgtaacccgtacatgcccaaaatagggggcgggttacacagaatatataacatcgtaggtgtctgggtgaacagtttattcctggcatccactaaatataatggagcccgctttttaagctggcatccagaaaaaaaaagaatcccagcaccaaaatattgttttcttcaccaaccatcagttcataggtccattctcttagcgcaactacagagaacaggggcacaaacaggcaaaaaacgggcacaacctcaatggagtgatgcaacctgcctggagtaaatgatgacacaaggcaattgacccacgcatgtatctatctcattttcttacaccttctattaccttctgctctctctgatttggaaaaagctgaaaaaaaaggttgaaaccagttccctgaaattattcccctacttgactaataagtatataaagacggtaggtattgattgtaattctgtaaatctatttcttaaacttcttaaattctacttttatagttagtcttttttttagttttaaaacaccaagaacttagtttcgaataaacacacataaacaaacaaagatgatgcagttacttcgctgtttttcaatattttctgttattgcttcagttttagcacaggaactgacaactatatgcgagcaaatcccctcaccaactttagaatcgacgccgtactctttgtcaacgactactattttggccaacgggaaggcaatgcaaggagtttttgaatattacaaatcagtaacgtttgtcagtaattgcggttctcacccctcaacaactagcaaaggcagccccataaacacacagtatgtttttaagcttctgcaggctagtggtggtggtggttctggtggtggtggttctggtggtggtggttctgctagcatgactggtggacagcaaatgggtcgggatctgtacgacgatgacgataaggtaccaggatccatgaagtgtacgttgaaatccttcactgtagaaaaaggaatctatcaaacttctaactttagagtccaaccaacagaatctattgttagatttcctaatattacaaacttgtgcccttttggtgaagtttttaacgccaccagatttgcatctgtttatgcttggaacaggaagagaatcagcaactgtgttgctgattattctgtcctatataattccgcatcattttccacttttaagtgttatggagtgtctcctactaaattaaatgatctctgctttactaatgtctatgcagattcatttgtaattagaggtgatgaagtcagacaaatcgctccagggcaaactggaaagattgctgattataattataaattaccagatgattttacaggctgcgttatagcttggaattctaacaatcttgattctaaggttggtggtaattataattacctgtatagattgtttaggaagtctaatctcaaaccttttgagagagatatttcaactgaaatctatcaggccggtagcacaccttgtaatggtgttgaaggttttaattgttactttcctttacaatcatatggtttccaacccactaatggtgttggttaccaaccatacagagtagtagtactttcttttgaacttctacatgcaccagcaactgtttgtggacctaaaaagtctactaatttggttaaaaacaaatgtgtcaatttcaacttcaatggtttaacaggcacaggtgttcttactgagtctaacaaaaagtttctgcctttccaacaatttggcagagacattgctgacactactgatgctgtccgtgatccacagacacttgagattcttgacattacaccatgttcttttggtggtgtcagtgttataacaccaggaacaaatacttctaaccaggttgctgttctttatcaggatgttaactgcacagaagtccctgttgctattcatgcagatcaacttactcctacttggcgtgtttattctacaggttctaatgtttttcaaacacgtgcaggctgtttaataggggctgaacatgtcaacaactcatatgagtgtgacatacccattggtgcaggtatatgcgctagttatcagactcagactaattctcctcggcgggcacgtagtgtagctagtcaatccatcattgcctacactatgtcacttggtgcagaaaattcagttgcttactctaataactctattgccatacccacaaattttactattagtgttaccacagaaattctaccagtgtctatgaccaagacatcagtagattgtacaatgtacatttgtggtgattcaactgaatgcagcaatcttttgttgcaatatggcagtttttgtacacaattaaaccgtgctttaactggaatagctgttgaacaagacaaaaacacccaagaagtttttgcacaagtcaaacaaatttacaaaacaccaccaattaaagattttggtggttttaatttttcacaaatattaccagatccatcaaaaccaagcaagaggtcatttattgaagatctacttttcaayaaagtgacacttgcagatgctggcttcatcaaacaatatggtgattgccttggtgatattgctgctagagacctcatttgtgcacaaaagtttaacggccttactgttttgccacctttgctcacagatgaaatgattgctcaatacacttctgcactgttagcgggtacaatcacttctggttggacctttggtgcaggtgctgcattacaaataccatttgctatgcaaatggcttataggtttaatggtattggagttacacagaatgttctctatgagaaccaaaaattgattgccaaccaatttaatagtgctattggcaaaattcaagactcactttcttccacagcaagtgcacttggaaaacttcaagatgtggtcaaccaaaatgcacaagctttaaacacgcttgttaaacaacttagctccaattttggtgcaatttcaagtgttttaaatgatatcctttcacgtcttgacaaagttgaggctgaagtgcaaattgataggttgatcacaggcagaggatccagtgtggtggaattctgcagatatccagcacagtggcggccgctcgagtctagagggcccttcgaaggtaagcctatccctaaccctctcctcggcctcgattctacgcgtaccggtcatcatcaccatcaccattgatagccgaatttcttatgatttatgatttttattattaaataagttataaaaaaaataagtgtatacaaattttaaagtgactcttaggttttaaaacgaaaattcttattcttgagtaactctttcctgtaggtcaggttgctttctcaggtatagcatgaggtcgctcttattgaccacacctctaccggcctctgagagagacccaagacactgcggatcgagaccactagtaccggtctgcagcgcgagggggggcccggtgcccaattcgccctatagtgagtcgtattacgcgcgctcactggccgtcgttttacaacgtcgtgactgggaaaaccctggcgttacccaacttaatcgccttgcagcacatccccctttcgccagctggcgtaatagcgaagaggcccgcaccgatcgcccttcccaacagttgcgcagcctgaatggcgaatggcgcgacgcgccctgtagcggcgcattaagcgcggcgggtgtggtggttacgcgcagcgtgaccgctacacttgccagcgccctagcgcccgctcctttcgctttcttcccttcctttctcgccacgttcgccggctttccccgtcaagctctaaatcgggggctccctttagggttccgatttagtgctttacggcacctcgaccccaaaaaacttgattagggtgatggttcacgtagtgggccatcgccctgatagacggtttttcgccctttgacgttggagtccacgttctttaatagtggactcttgttccaaactggaacaacactcaaccctatctcggtctattcttttgatttataagggattttgccgatttcggcctattggttaaaaaatgagctgatttaacaaaaatttaacgcgaattttaacaaaatattaacgtttacaatttcctgatgcggtattttctccttacgcatctgtgcggtatttcacaccgcatagggtaataactgatataattaaattgaagctctaatttgtgagtttagtatacatgcatttacttataatacagttttttagttttgctggccgcatcttctcaaatatgcttcccagcctgcttttctgtaacgttcaccctctaccttagcatcccttccctttgcaaatagtcctcttccaacaataataatgtcagatcctgtagacaccacatcatccacggttctatactgttgacccaatgcgtcacccttgtcatctaaacccacaccgggtgtcataatcaaccaatcgtaaccttcatctcttccacccatgtctctttgagcaataaagccgataacaaaatctttgtcgctcttcgcaatgtcaacagtacccttagtatattctccagtagatagggagcccttgcatgacaattctgctaacatcaaaaggcctctaggttcctttgttacttcttctgccgcctgcttcaaaccgctaacaatacctgggcccaccacaccgtgtgcattcgtaatgtctgcccattctgctattctgtatacacccgcagagtactgcaatttgactgtattaccaatgtcagcaaattttctgtcttcgaagagtaaaaaattgtacttggcggataatgcctttagcggcttaactgtgccctccatggaaaaatcagtcaagatatccacatgtgtttttagtaaacaaattttgggacctaatgcttcaactaactccagtaattccttggtggtacgaacatccaatgaagcacacaagtttgtttgcttttcgtgcatgatattaaatagcttggcagcaacaggactaggatgagtagcagcacgttccttatatgtagctttcgacatgatttatcttcgtttcctgcaggtttttgttctgtgcagttgggttaagaatactgggcaatttcatgtttcttcaacactacatatgcgtatatataccaatctaagtctgtgctccttccttcgttcttccttctgttcggagattaccgaatcaaaaaaatttcaaagaaaccgaaatcaaaaaaaagaataaaaaaaaaatgatgaattgaattgaaaagctgtggtatggtgcactctcagtacaatctgctctgatgccgcatagttaagccagccccgacacccgccaacacccgctgacgcgccctgacgggcttgtctgctcccggcatccgcttacagacaagctgtgacaatctccgggagctgcatgtgtcagaggttttcaccgtcatcaccgaaacgcgcgagattaa

SEQ ID NO: 4 - DNA, 43 bp, Artificial Synthesis
gacgataaggtaccaggatccatgaagtgtacgttgaaatcct

SEQ ID NO: 5 - DNA, 41 bp, Artificial Synthesis
gaattccaccacactggatcctctgcctgtgatcaacctat

SEQ ID NO: 6 - DNA, 21 bp, Artificial Synthesis
aatattacaaacttgtgccct

SEQ ID NO: 7 - DNA, 21 bp, Artificial Synthesis
aacagttgctggtgcatgtag